European Patent Specification EP 3 127 914 B1, published December 17, 2025. Title: Long term functional adrenomedullin derivative. Applicant: University of Miyazaki. The sequence listing filed with the application follows.

SEQUENCE LISTING (12 sequences)

SEQ ID NO: 1 - protein, 52 aa, Homo sapiens
YRQSMNNFQGLRSFGCRFGTCTVQKLAHQIYQFTDKDKDNVAPRSKISPQGY

SEQ ID NO: 2 - DNA, 1449 bp, Homo sapiens
  CDS (157)..(711)
ctggatagaacagctcaagccttgccacttcgggcttctcactgcagctgggcttggacttcggagttttgccattgccagtgggacgtctgagactttctccttcaagtacttggcagatcactctcttagcagggtctgcgcttcgcagccgggatgaagctggtttccgtcgccctgatgtacctgggttcgctcgccttcctaggcgctgacaccgctcggttggatgtcgcgtcggagtttcgaaagaagtggaataagtgggctctgagtcgtgggaagagggaactgcggatgtccagcagctaccccaccgggctcgctgacgtgaaggccgggcctgcccagacccttattcggccccaggacatgaagggtgcctctcgaagccccgaagacagcagtccggatgccgcccgcatccgagtcaagcgctaccgccagagcatgaacaacttccagggcctccggagctttggctgccgcttcgggacgtgcacggtgcagaagctggcacaccagatctaccagttcacagataaggacaaggacaacgtcgcccccaggagcaagatcagcccccagggctacggccgccggcgccggcgctccctgcccgaggccggcccgggtcggactctggtgtcttctaagccacaagcacacggggctccagcccccccgagtggaagtgctccccactttctttaggatttaggcgcccatggtacaaggaatagtcgcgcaagcatcccgctggtgcctcccgggacgaaggacttcccgagcggtgtggggaccgggctctgacagccctgcggagaccctgagtccgggaggcaccgtccggcggcgagctctggctttgcaagggcccctccttctgggggcttcgcttccttagccttgctcaggtgcaagtgccccagggggcggggtgcagaagaatccgagtgtttgccaggcttaaggagaggagaaactgagaaatgaatgctgagacccccggagcaggggtctgagccacagccgtgctcgcccacaaactgatttctcacggcgtgtcaccccaccagggcgcaagcctcactattacttgaactttccaaaacctaaagaggaaaagtgcaatgcgtgttgtacatacagaggtaactatcaatatttaagtttgttgctgtcaagattttttttgtaacttcaaatatagagatatttttgtacgttatatattgtattaagggcattttaaaagcaattatattgtcctcccctattttaagacgtgaatgtctcagcgaggtgtaaagttgttcgccgcgtggaatgtgagtgtgtttgtgtgcatgaaagagaaagactgattacctcctgtgtggaagaaggaaacaccgagtctctgtataatctatttacataaaatgggtgatatgcgaacagcaaacc

SEQ ID NO: 3 - protein, 52 aa, Sus scrofa
YRQSMNNFQGLRSFGCRFGTCTVQKLAHQIYQFTDKDKDGVAPRSKISPQGY

SEQ ID NO: 4 - DNA, 1493 bp, Sus scrofa
gcggaacagctcgagccttgccacctctagtttcttaccacagcttggacgtcggggttttgccactgccagagggacgtctcagacttcatcttcccaaatcttggcagatcacccccttagcagggtctgcacatctcagccgggatgaagctggttcccgtagccctcatgtacctgggctcgctcgccttcctgggcgctgacacagctcggctcgacgtggcggcagagttccgaaagaaatggaataagtgggctctaagtcgtggaaaaagagaacttcggctgtccagcagctaccccaccgggatcgccgacttgaaggccgggcctgcccagactgtcattcggccccaggatgtgaagggctcctctcgcagcccccaggccagcattccggatgcagcccgcatccgagtcaagcgctaccgccagagtatgaacaacttccagggcctgcggagcttcggctgtcgctttgggacgtgcaccgtgcagaagctggcgcaccagatctaccagttcacggacaaagacaaggacggcgtcgccccccggagcaagatcagcccccagggctacggccgccggcgccgacgctctctgcccgaagccagcctgggccggactctgaggtcccaggagccacaggcgcacggggccccggcctccccggcgcatcaagtgctcgccactctctttaggatttaggcgcctactgtggcagcagcgaacagtcgcgcatgcatcatgccggcgcttcctggggcggggggcttcccggagccgagcccctcagcggctggggcccgggcagagacagcattgagagaccgagagtccgggaggcacagaccagcggcgagccctgcattttcaggaacccgtcctgcttggaggcagtgttctcttcggcttaatccagcccgggtccccgggtgggggtggagggtgcagaggaatccaaaggagtgtcatctgccaggctcacggagaggagaaactgcgaagtaaatgcttagacccccaggggcaagggtctgagccactgccgtgccgcccacaaactgatttctgaaggggaataaccccaacagggcgcaagcctcactattacttgaactttccaaaacctagagaggaaaagtgcaatgtatgttgtatataaagaggtaactatcaatatttaagtttgttgctgtcaagatttttttttgtaacttcaaatatagagatatttttgtacgttatatattgtattaagggcattttaaaacaattgtattgttcccctcccctctattttaatatgtgaatgtctcagcgaggtgtaacattgtttgctgcgcgaaatgtgagagtgtgtgtgtgtgtgtgcgtgaaagagagtctggatgcctcttggggaagaagaaaacaccatatctgtataatctatttacataaaatgggtgatatgcgaagtagcaaaccaataaactgtctcaatg

SEQ ID NO: 5 - protein, 52 aa, Canis familiaris
YRQSMNNFQGPRSFGCRFGTCTVQKLAHQIYQFTDKDKDGVAPRSKISPQGY

SEQ ID NO: 6 - DNA, 1432 bp, Canis familiaris
ggttttgccagcaccagagcgacgtctcagaccttctcctcccggatcttggcagatcaccccctcagcagggtctgcgcatcgccgccagcatgaagctggttcccgtcgccctcttatacctgggctccctcgccttcttgggcgcggacaccgcacggctagacgtggcgtcagagttccgaaagaagtggaataaatgggctgtaagtcgtggaaagagggaacttcgagtgtccagcagctatcccaccgggctcgctgaagtgaaggccgggccggcccagactcttattcggacccaggacgtgaagggcgcctctcgcaacccccagaccagcggtccggacgccgcccgcatccgagtcaaacgctaccgccagagtatgaacaatttccagggcccgcggagcttcggctgccgcttcggaacgtgcacggtgcagaaactggcgcaccagatctaccagttcacagacaaggacaaggacggcgtcgcccccaggagcaagattagccctcagggctacggccgccggcgccggcgctccctgcccgagcccggccttcgccggactctgttgttcccggagccacggccaggcggggctccggccccccgggcgcatcaggtgctcgccaacctccttaagatgtaggcgcctgtggcagcagcgaactggcgcgcgtgtgcatcccgctggcttccccctgggcggagggcttccccgagccgagcccctctgccgatggaagtcgggcagagaccgggattccgggaggcaccgtcccgcggccagccctggctttgcgcgagccccttctcctcggaggcacggatccctctgtcccaagccggcccaggtgtcccgtggggggcagaggaatgcaagggaggcctgccaggctcacggagaggattaactgagaattaaatgagaattaaatgcttgagaccctcccccctccccccccagggacaggggtctgagtcactgccgtgcctgcccacaaactgatttctcacggggtgtcaccccaccggggcgcaagcctcactattacttgaactttccaaaacctagagaggaaaagtgcaatgcgtgttgtatatacagaggtaactatcaatatttaagttcgttgctgtcagaagattttttttgtaacttcaaatatagagatatttttgtacgttatatattgtattaagggcatttaaaaaccattgcattgtccccctccccacttattttaatacgtgaatgtctcagcgaggtgtaacgttgtttttgctgcagagtgtgtgagtgtgcgtgagagacttattacctcttgtggaagaaggaacaccgtgtctctgcattatctatttacataaaatgggtgatatgcgaaaatagcaaatcaataataaacggtctcgatgctg

SEQ ID NO: 7 - protein, 52 aa, Bos taurus
YRQSLNNFQGLRSFGCRFGTCTVQKLAHQIYHFTDKDKDGSAPRSKISPQGY

SEQ ID NO: 8 - DNA, 1439 bp, Bos taurus
cgggaaacagctcgaaccttctcacttttggcttctcactgcagcttcgacgtcggggttttgccactgccagaacgccgtctcagacttaatactccaaagaattttggcagatcaccccctcagcagggtctgcgcatcgccgccgggatgaagctggttcccgtcgccctcctgtacctggggtcgctcgccttcctaggcgtggacacggcacggctcgacgtggcggcagagttccgaaagaaatggaataagtgggctctaagtcgtggaaaaagagaacttcgcgagtccagtagctaccccaccgggctcgccgacgtgaaggccgggcctgtccagactcttattcggccccaggatgtaaagggcgcctctcgaagccctcaggccagcagtcctgacgcagcccgcatccgagtcaagcgctaccgccagagtttgaacaacttccagggcctgcggagcttcggttgtcgcttcgggacatgcacggtgcagaagttggcgcatcagatctaccatttcacggacaaggacaaggacggatccgcccccaggagcaagatcagcccccagggctacggccgtcggcgccgacgttcactgcctgaggccggcttgggtcggactctattacagcctccagagccaaagctgcgaggggccccggactcccgggtgcatcaagtacttgccaccctcaggatttaggcgcctgggcagcagcgaacagtcgcgcacgcatctcgccggcacctcttcgggcgggagggcttccgcgagccgagcccctcactcagcctatgggcccgggctgagaacagccctgagagaccgagagtccaggaggcaccgtccggcagccagcgagcactggctttgcaggaacccgtcctcctcggaggggaggcagtgttctcttcactctaattggggccaggtgcagtttctcctctccgtgagcctggcagacgctcacggagaggagaaactgcgaaataaatgatgagaccctcaggggcaagggtctgagccactgccgtgcccgcccacaaactgattcctgatgggggtgtcaccccaccggggtgcaagcctcactattacttgaactttccgaaacctagagaggaaaagtgcaatgagtgttgtatatacagagataattatcaatatttaaatttgttgttgtcaagattttttttgtaacttcaaatatagagatatttttgtacgttatatattgtattaagggcattttaaagcaattgtattgttcccctcccctctattttaataagtgaatgtctcagcgagatgcaacgttgtttgctgcgtggaatgtgagagtgtgtgcgtgaaagagatgagttgcctcttgtggaagaagaaaacaccgtgtctgtataatctatttacataaagtgggccgg

SEQ ID NO: 9 - protein, 50 aa, Rattus norvegicus
YRQSMNQGSRSTGCRFGTCTMQKLAHQIYQFTDKDKDGMAPRNKISPQGY

SEQ ID NO: 10 - DNA, 1376 bp, Rattus norvegicus
tccagcctttaccgctcctggtttctcggcttctcatcgcagtcagtcttggactttgcgggttttgccgctgtcagaaggacgtctcggactttctgcttcaagtgcttgacaactcaccctttcagcagggtatcggagcatcgctacagaatgaagctggtttccatcgccctgatgttattgggttcgctcgccgttctcggcgcggacaccgcacggctcgacacttcctcgcagttccgaaagaagtggaataagtgggcgctaagtcgtgggaagagggaactacaagcgtccagcagctaccctacggggctcgttgatgagaagacagtcccgacccagactcttgggctccaggacaagcagagcacgtctagcaccccacaagccagcactcagagcacagcccacattcgagtcaaacgctaccgccagagcatgaaccaggggtcccgcagcactggatgccgctttgggacctgcacaatgcagaaactggctcaccagatctaccagtttacagacaaagacaaggacggcatggcccccagaaacaagatcagccctcaaggctatggccgccggcgccggcgttccctgccagaggtcctccgagcccggactgtggagtcctcccaggagcagacacactcagctccagcctccccggcgcaccaagacatctccagagtctctaggttataggtgcgggtggcagcattgaacagtcgggcgagtatcccattggcgcctgcggaatcagagagcttcgcaccctgagcggactgagacaatcttgcagagatctgcctggctgcccctaggggaggcagaggaacccaagatcaagccaggctcacgtcagaaaccgagaattacaggctgatactctctccgggcaggggtctgagccactgccttgcccgctcataaactggttttctcacggggcatacggctcattacttacttgaactttccaaaacctagcgaggaaaagtgcaatgcttgttatacagccaaaggtaactatcatatttaagtttgttgatgtcaagaggtttttttttttgtaacttcaaatatatagaaatatttttgtacgttatatattgtattaagggcattttaaagcgattatattgtcaccttcccctattttaagaagtgaatgtctcagcaaggtgtaaggttgtttggttccgtgtgtgtgtgtgtgtgtgtgtgtgtgtgtgtgtgtgtgtgtgtgtaaggtggagagcgcctgattaccgcctgtggatgaagaaaaaacattgtgtcttctataatctatttacataaaatatgtgatctgggaaaaagcaaaccaataaactgtctcaatgctg

SEQ ID NO: 11 - protein, 50 aa, Mus musculus
YRQSMNQGSRSNGCRFGTCTFQKLAHQIYQLTDKDKDGMAPRNKISPQGY

SEQ ID NO: 12 - DNA, 1381 bp, Mus musculus
cttggtgacactagacagagcaactccagcgttaccgctcccgctcctggtttctcggcttctcatcgcagtcaatcttggactttggggttttgctactgtcagaaggacttctttctgcttcaagtgcttgacaacgcacccctttatcagggtatcagagcatcgccacagaatgaagctggtttccatcaccctgatgttattgggttcactcgctttcctaggcgcggacactgcagggccagatactccttcgcagttccgaaagaagtggaataagtgggcgctaagtcgtgggaagagggaactacaagcatccagcagctaccctacgggactcgctgatgagacgacagttcctacccagactcttgatccattcctggacgagcagaacacaactggccccctacaagccagcaatcagagcgaagcccacattcgtgtcaaacgctaccgccagagcatgaaccagggttcccgcagcaatggatgccgcttcgggacctgcacatttcagaaattggcccaccagatctaccagctaacagacaaagacaaggacggcatggctcccagaaacaagatcagccctcaaggctatggccgccggcgccggcgttccctgctggaggtcctccggtcccggactgtggagtcctcccaggagcagacacacacagccccaggcccctgggcgcacatctccagactctttaggatataggtgcgggtgacagcattgaacagtcgggcgagtatcccgttggcgcctgcggaatcagagaacttcgcaccggggcggactgagacaatcctgcagagatctgcctggctgcccctaggggaggcagaggaacccaagaccaagccaggctcatgccagaaaccgagacttacaggctgatactctccgggcaggggtctgagccactgccttgcccgctcataaactggtttctcacggggcataagcctcattactacttgaactttccaaaacctagcgaggaacgtgcaatgcttgttgtccagccaaaggtaactatagtatttaagtttgttgctgtcaaggtttttttttttgtaacttcaaatatatagagatatttttgtacgttatatattgtattaagggcattttaaagtgattatattgtcaccttcccctattttaagacgtgaatgtctcagcaaggtgtaaggttgtttggttccgtgtgtgtgtgtgtgtgtgtgtgtgtgtgtgtgtgtgtgtaaggtggagagcgcctgattatcgcctgtggatgaagaaaaaacattgtgtttcctataatctatttacataaaatatgtgatctgggaaaaagcaaaccaataaactgtctcaatgctg